European Patent Specification EP 3 710 594 B1, published July 19, 2023. Title: METHODS TO MEASURE FUNCTIONAL HETEROGENEITY AMONG SINGLE CELLS. Applicant: The Regents of the University of Colorado, a body corporate Hesselberth, Jay. Application Not yet assigned. The sequence listing filed with the application follows.

SEQUENCE LISTING (8 sequences)

SEQ ID NO: 1 - DNA, 8 bp, Artificial Sequence
  Synthetic
atgctagc

SEQ ID NO: 2 - DNA, 8 bp, Artificial Sequence
  Synthetic
taggctta

SEQ ID NO: 3 - DNA, 8 bp, Artificial Sequence
  Synthetic
taggtcaa

SEQ ID NO: 4 - DNA, 9 bp, Artificial Sequence
  Synthetic
gatcgtagc

SEQ ID NO: 5 - DNA, 9 bp, Artificial Sequence
  Synthetic
aatcgatct

SEQ ID NO: 6 - DNA, 9 bp, Artificial Sequence
  Synthetic
ttccgatat

SEQ ID NO: 7 - DNA, 6 bp, Artificial Sequence
  Synthetic
aaaaaa

SEQ ID NO: 8 - DNA, 6 bp, Artificial Sequence
  Synthetic
tttttt